European Patent Application EP 4 349 985 A1, published April 10, 2024. Title: PEPTIDE TRANSLATED BY CIRCULAR RNA CIRC-ACE2 AND APPLICATION THEREOF. Applicant: GUANGZHOU INSTITUTES OF BIOMEDICINE AND HEALTH, CHINESE ACADEMY OF SCIENCES. The sequence listing filed with the application follows.

SEQUENCE LISTING (7 sequences)

SEQ ID NO: 1 - RNA, 289 nt, synthetic construct
  source 1..289: mol_type = other RNA
cgcccaacccaagttcaaaggctgataagagagaaaatctcatgaggaggttttagtctagggaaagtcattcagtggatgtgatcttggctcacaggggacgatgtcaagctcttcctggctccttctcagccttgttgctgtaactgctgctcagtccaccattgaggaacaggccaagacatttttggacaagtttaaccacgaagccgaagacctgttctatcaaagttcacttgcttcttggaattataacaccaatattactgaagagaatgtccaaaacatg

SEQ ID NO: 2 - RNA, 231 nt, synthetic construct
  source 1..231: mol_type = other RNA
atgtcaagctcttcctggctccttctcagccttgttgctgtaactgctgctcagtccaccattgaggaacaggccaagacatttttggacaagtttaaccacgaagccgaagacctgttctatcaaagttcacttgcttcttggaattataacaccaatattactgaagagaatgtccaaaacatgcgcccaacccaagttcaaaggctgataagagagaaaatctcatga

SEQ ID NO: 3 - protein, 76 aa, synthetic construct
MSSSSWLLLSLVAVTAAQSTIEEQAKTFLDKFNHEAEDLFYQSSLASWNYNTNITEENVQNMRPTQVQRLIREKIS

SEQ ID NO: 4 - protein, 320 aa, synthetic construct
MSSSSWLLLSLVAVTAAQSTIEEQAKTFLDKFNHEAEDLFYQSSLASWNYNTNITEENVQNMRPTQVQRLIREKISLVPRGSGGGGDPEPKSCDKTHTCPPCPAPELLGGPSVFLFPPKPKDTLMISRTPEVTCVVVDVSHEDPEVKFNWYVDGVEVHNAKTKPREEQYNSTYRVVSVLTVLHQDWLNGKEYKCKVSNKALPAPIEKTISKAKGQPREPQVYTLPPSRDELTKNQVSLTCLVKGFYPSDIAVEWESNGQPENNYKTTPPVLDSDGSFFLYSKLTVDKSRWQQGNVFSCSVMHEALHNHYTQKSLSLSPGK

SEQ ID NO: 5 - DNA, 963 bp, synthetic construct
  source 1..963: mol_type = other DNA
atgtcaagctcttcctggctccttctcagccttgttgctgtaactgctgctcagtccaccattgaggaacaggccaagacatttttggacaagtttaaccacgaagccgaagacctgttctatcaaagttcacttgcttcttggaattataacaccaatattactgaagagaatgtccaaaacatgcgcccaacccaagttcaaaggctgataagagagaaaatctcactggtgcccagaggctccggcggcggcggcgatcctgagcccaaatcttgtgacaaaactcacacatgcccaccgtgcccagcacctgaactcctggggggaccgtcagtcttcctcttccccccaaaacccaaggacaccctcatgatctcccggacccctgaggtcacatgcgtggtggtggacgtgagccacgaagaccctgaggtcaagttcaactggtacgtggacggcgtggaggtgcataatgccaagacaaagccgcgggaggagcagtacaacagcacgtaccgtgtggtcagcgtcctcaccgtcctgcaccaggactggctgaatggcaaggagtacaagtgcaaggtctccaacaaagccctcccagcccccatcgagaaaaccatctccaaagccaaagggcagccccgagaaccacaggtgtacaccctgcccccatcccgggatgagctgaccaagaaccaggtcagcctgacctgcctggtcaaaggcttctatcccagcgacatcgccgtggagtgggagagcaatgggcagccggagaacaactacaagaccacgcctcccgtgctggactccgacggctccttcttcctctacagcaagctcaccgtggacaagagcaggtggcagcaggggaacgtcttctcatgctccgtgatgcatgaggctctgcacaaccactacacgcagaagagcctctccctgtctccgggtaaatga

SEQ ID NO: 6 - protein, 59 aa, synthetic construct
QSTIEEQAKTFLDKFNHEAEDLFYQSSLASWNYNTNITEENVQNMRPTQVQRLIREKIS

SEQ ID NO: 7 - DNA, 1132 bp, synthetic construct
  source 1..1132: mol_type = other DNA
agtgctgagattacaggcgtgagccaccacccccggcccactttttgtaaaggtacgtactaatgactttttttttatacttcagcgcccaacccaagttcaaaggctgataagagagaaaatctcaaagggcgaggaggataacatggccatcatcaaggagttcatgcgcttcaaggtgcacatggagggctccgtgaacggccacgagttcgagatcgagggcgagggcgagggccgcccctacgagggcacccagaccgccaagctgaaggtgaccaagggtggccccctgcccttcgcctgggacatcctgtcccctcagttcatgtacggctccaaggcctacgtgaagcaccccgccgacatccccgactacttgaagctgtccttccccgagggcttcaagtgggagcgcgtgatgaacttcgaggacggcggcgtggtgaccgtgacccaggactcctccctgcaggacggcgagttcatctacaaggtgaagctgcgcggcaccaacttcccctccgacggccccgtaatgcagaagaagactatgggctgggaggcctcctccgagcggatgtaccccgaggacggcgccctgaagggcgagatcaagcagaggctgaagctgaaggacggcggccactacgacgctgaggtcaagaccacctacaaggccaagaagcccgtgcagctgcccggcgcctacaacgtcaacatcaagttggacatcacctcccacaacgaggactacaccatcgtggaacagtacgaacgcgccgagggccgccactccaccggcggcatggacgagctgtacaagtgaggaggttttagtctagggaaagtcattcagtggatgtgatcttggctcacaggggacgatgtcaagctcttcctggctccttctcagccttgttgctgtaactgctgctcagtccaccattgaggaacaggccaagacatttttggacaagtttaaccacgaagccgaagacctgttctatcaaagttcacttgcttcttggaattataacaccaatattactgaagagaatgtccaaaacatggtaagaagcaaggaaaagaattaggctcggcacggtagctcacacctgtaatcccagca